European Patent Specification EP 3 375 450 B1, published June 28, 2023. Title: Composition for Treatment of Brain Stroke by Intranasal Delivery. Applicant: IUCF-HYU (Industry-University Cooperation Foundation Hanyang University). The sequence listing filed with the application follows.

SEQUENCE LISTING (2 sequences)

SEQ ID NO: 1 - protein, 8 aa, Artificial Sequence
  Fas targeting peptide
YCDEHFCY

SEQ ID NO: 2 - protein, 8 aa, Artificial Sequence
  Scrambled peptide
YCNSTVCY